European Patent Application EP 4 685 144 A1, published January 28, 2026. Title: NON-FLUORESCENT COMPOUND AND THEIR APPLICATIONS. Applicant: SFC CO., LTD. Application KR. The sequence listing filed with the application follows.

SEQUENCE LISTING (14 sequences)

SEQ ID NO: 1 - DNA, 10 bp, synthetic construct
  source 1..10: mol_type = other DNA; note = oligonucleotide used in Experimental Example 1
tttttttttt

SEQ ID NO: 2 - DNA, 30 bp, synthetic construct
  source 1..30: mol_type = other DNA; note = oligonucleotide for forward probe used in Experimental Example 2 and 3
tttttttttttagcttgcagatgtcatagt

SEQ ID NO: 3 - DNA, 30 bp, synthetic construct
  source 1..30: mol_type = other DNA; note = oligonucleotide for reverse probe used in Experimental Example 2 and 3
actatgacatctgcaagctaaaaaaaaaaa

SEQ ID NO: 4 - DNA, 25 bp, synthetic construct
  source 1..25: mol_type = other DNA; note = oligonucleotide for reverse probe used in Experimental Example 2
actatgacatctgcaagctaaaaaa

SEQ ID NO: 5 - DNA, 20 bp, synthetic construct
  source 1..20: mol_type = other DNA; note = oligonucleotide for reverse probe used in Experimental Example 2
actatgacatctgcaagcta

SEQ ID NO: 6 - DNA, 23 bp, synthetic construct
  source 1..23: mol_type = other DNA; note = Black queen cell virus complement
ccatctttatcggtacgccgccc

SEQ ID NO: 7 - DNA, 23 bp, synthetic construct
  source 1..23: mol_type = other DNA; note = Neisseria gonorrhoeae complement
cagtcgagaacagcaaagcaacg

SEQ ID NO: 8 - DNA, 28 bp, synthetic construct
  source 1..28: mol_type = other DNA; note = Mycoplasma genitalium complement
agcctttctaaccgctgcacttaccctt

SEQ ID NO: 9 - DNA, 27 bp, synthetic construct
  source 1..27: mol_type = other DNA; note = Chlamydia trachomatis complement
ttgtccatatctttgatacgacgccgc

SEQ ID NO: 10 - DNA, 20 bp, synthetic construct
  source 1..20: mol_type = other DNA; note = oligonucleotide used in Experimental Example6
tttttttttttttttttttt

SEQ ID NO: 11 - DNA, 14 bp, synthetic construct
  source 1..14: mol_type = other DNA; note = Black queen cell virus complement
ttatcggtacgccg

SEQ ID NO: 12 - DNA, 36 bp, synthetic construct
  source 1..36: mol_type = other DNA; note = n refers to the Quencher (Eclipse) inserted between oligonucleotides
aagagtagtnagcctaagagtgtcagttgtacatca

SEQ ID NO: 13 - DNA, 35 bp, synthetic construct
  source 1..35: mol_type = other DNA; note = oligonucleotide used in Experimental Example8
aagagtagtagcctaagagtgtcagttgtacatca

SEQ ID NO: 14 - DNA, 36 bp, synthetic construct; identical to SEQ ID NO: 12
  source 1..36: mol_type = other DNA; note = n refers to the Quencher (ZEN) inserted between oligonucleotides